European Patent Application EP 4 299 745 A1, published January 3, 2024. Title: Anti-SARS-CoV-2 antibody. Applicant: KAO CORPORATION EPSILON MOLECULAR ENGINEERING, INC. The sequence listing filed with the application follows.

SEQUENCE LISTING (51 sequences)

SEQ ID NO: 1 - protein, 10 aa, Artificial Sequence
  Designed peptide
GFPFTKFWMY

SEQ ID NO: 2 - protein, 10 aa, Artificial Sequence
  Designed peptide
FIDTTGTITN

SEQ ID NO: 3 - protein, 13 aa, Artificial Sequence
  Designed peptide
GPPGSTWVVDFHS

SEQ ID NO: 4 - protein, 10 aa, Artificial Sequence
  Designed peptide
GFTFDDHAVG

SEQ ID NO: 5 - protein, 10 aa, Artificial Sequence
  Designed peptide
AISGDGYTTV

SEQ ID NO: 6 - protein, 9 aa, Artificial Sequence
  Designed peptide
FRTDIVREY

SEQ ID NO: 7 - protein, 26 aa, Artificial Sequence
  Designed peptide
AEVQLVESGGAVVQPGGSLRLSCEAS

SEQ ID NO: 8 - protein, 26 aa, Artificial Sequence
  Designed peptide
AEVQLVESGGGSVQAGGSLTLSCAAS

SEQ ID NO: 9 - protein, 14 aa, Artificial Sequence
  Designed peptide
WVRRAPGKGLEWVA

SEQ ID NO: 10 - protein, 14 aa, Artificial Sequence
  Designed peptide
WFRQAPGKGLEWVS

SEQ ID NO: 11 - protein, 39 aa, Artificial Sequence
  Designed peptide
YASSVKGRFTISRDDARNMVYLQMNDLRPEDTAIYYCAT

SEQ ID NO: 12 - protein, 39 aa, Artificial Sequence
  Designed peptide
YADSVKGRFTISRDNAKKTVYLQMNSLKAEDTAVYYCNA

SEQ ID NO: 13 - protein, 11 aa, Artificial Sequence
  Designed peptide
WGQGTQVTVSS

SEQ ID NO: 14 - protein, 123 aa, Artificial Sequence
  Designed peptide
AEVQLVESGGAVVQPGGSLRLSCEASGFPFTKFWMYWVRRAPGKGLEWVAFIDTTGTITNYASSVKGRFTISRDDARNMVYLQMNDLRPEDTAIYYCATGPPGSTWVVDFHSWGQGTQVTVSS

SEQ ID NO: 15 - protein, 119 aa, Artificial Sequence
  Designed peptide
AEVQLVESGGGSVQAGGSLTLSCAASGFTFDDHAVGWFRQAPGKGLEWVSAISGDGYTTVYADSVKGRFTISRDNAKKTVYLQMNSLKAEDTAVYYCNAFRTDIVREYWGQGTQVTVSS

SEQ ID NO: 16 - DNA, 33 bp, Artificial Sequence
  Synthetic oligonucleotide
gatcccgcgaaattaatacgactcactataggg

SEQ ID NO: 17 - DNA, 22 bp, Artificial Sequence
  Synthetic oligonucleotide
tttccacgccgccccccgtcct

SEQ ID NO: 18 - DNA, 60 bp, Artificial Sequence
  Synthetic oligonucleotide
gatcccgcgaaattaatacgactcactataggggaagtatttttacaacaattaccaaca

SEQ ID NO: 19 - DNA, 58 bp, Artificial Sequence
  Synthetic oligonucleotide
  misc_feature (34)..(37): n is a, c, g, or t
tcgtcggcagcgtcagatgtgtataagagacagnnnnatggctgaggtgcagctcgtg

SEQ ID NO: 20 - DNA, 63 bp, Artificial Sequence
  Synthetic oligonucleotide
  misc_feature (35)..(38): n is a, c, g, or t
gtctcgtgggctcggagatgtgtataagagacagnnnntgatgatgatggctaccacctcccg

SEQ ID NO: 21 - protein, 123 aa, Artificial Sequence
  Designed peptide
AEVQLVESGGAVVQPGGSLRLSCEASGFPFTNFWMYWVRRAPGKGLEWVAFIDTTGTITNYASSVKGRFTISRDDARNMVYLQMNDLRPEDTAIYYCATGPPGSTWVVDFHSWGQGTQVTVSS

SEQ ID NO: 22 - protein, 123 aa, Artificial Sequence
  Designed peptide
AEVQLVESGGAVVQPGGSLRLSCEASGFPFTKLWMYWVRRAPGKGLEWVAFIDTTGTITNYASSVKGRFTISRDDARNMVYLQMNDLRPEDTAIYYCATGPPGSTWVVDFHSWGQGTQVTVSS

SEQ ID NO: 23 - protein, 123 aa, Artificial Sequence
  Designed peptide
AEVQLVESGGAVVQPGGSLRLSCEASGFPLTKFWMYWVRRAPGKGLEWVAFIDTTGTITNYASSVKGRFTISRDDARNMVYLQMNDLRPEDTAIYYCATGPPGSTWVVDFHSWGQGTQVTVSS

SEQ ID NO: 24 - protein, 123 aa, Artificial Sequence
  Designed peptide
AEVQLVESGGAVVQPGGSLRLSCEASGLPFTKFWMYWVRRAPGKGLEWVAFIDTTGTITNYASSVKGRFTISRDDARNMVYLQMNDLRPEDTAIYYCATGPPGSTWVVDFHSWGQGTQVTVSS

SEQ ID NO: 25 - protein, 123 aa, Artificial Sequence
  Designed peptide
AEVQLVESGGAVVQPGGSLRLSCEASGFPFTKFWVYWVRRAPGKGLEWVAFIDTTGTITNYASSVKGRFTISRDDARNMVYLQMNDLRPEDTAIYYCATGPPGSTWVVDFHSWGQGTQVTVSS

SEQ ID NO: 26 - protein, 123 aa, Artificial Sequence
  Designed peptide
AEVQLVESGGAVVQPGGSLRLSCEASGFPFTKFWRYWVRRAPGKGLEWVAFIDTTGTITNYASSVKGRFTISRDDARNMVYLQMNDLRPEDTAIYYCATGPPGSTWVVDFHSWGQGTQVTVSS

SEQ ID NO: 27 - protein, 123 aa, Artificial Sequence
  Designed peptide
AEVQLVESGGAVVQPGGSLRLSCEASRFPFTKFWMYWVRRAPGKGLEWVAFIDTTGTITNYASSVKGRFTISRDDARNMVYLQMNDLRPEDTAIYYCATGPPGSTWVVDFHSWGQGTQVTVSS

SEQ ID NO: 28 - protein, 123 aa, Artificial Sequence
  Designed peptide
AEVQLVESGGAVVQPGGSLRLSCEASGFPFTKCWMYWVRRAPGKGLEWVAFIDTTGTITNYASSVKGRFTISRDDARNMVYLQMNDLRPEDTAIYYCATGPPGSTWVVDFHSWGQGTQVTVSS

SEQ ID NO: 29 - protein, 123 aa, Artificial Sequence
  Designed peptide
AEVQLVESGGAVVQPGGSLRLSCEASGFPFTKFCMYWVRRAPGKGLEWVAFIDTTGTITNYASSVKGRFTISRDDARNMVYLQMNDLRPEDTAIYYCATGPPGSTWVVDFHSWGQGTQVTVSS

SEQ ID NO: 30 - protein, 123 aa, Artificial Sequence
  Designed peptide
AEVQLVESGGAVVQPGGSLRLSCEASGFPFTKFWMYWVRRAPGKGLEWVALIDTTGTITNYASSVKGRFTISRDDARNMVYLQMNDLRPEDTAIYYCATGPPGSTWVVDFHSWGQGTQVTVSS

SEQ ID NO: 31 - protein, 123 aa, Artificial Sequence
  Designed peptide
AEVQLVESGGAVVQPGGSLRLSCEASGFPFTKFWMYWVRRAPGKGLEWVAFIDTTGTITDYASSVKGRFTISRDDARNMVYLQMNDLRPEDTAIYYCATGPPGSTWVVDFHSWGQGTQVTVSS

SEQ ID NO: 32 - protein, 123 aa, Artificial Sequence
  Designed peptide
AEVQLVESEGAVVQPGGSLRLSCEASGFPFTKFWMYWVRRAPGKGLEWVAFIDTTGTITDYASSVKGRFTISRDDARNMVYLQMNDLRPEDTAIYYCATGPPGSTWVVDFHSWGQGTQVTVSS

SEQ ID NO: 33 - protein, 123 aa, Artificial Sequence
  Designed peptide
AEVQLVESGGAVVQPGGSLRLSCEASGFPFTKFWMYWVRRAPGKGLEWVAFIDTTGTITNYASSVKGRFTISRDDARNMVYLQMNDLRPEDTAIYYCATGPPGSTWVIDFHSWGQGTQVTVSS

SEQ ID NO: 34 - protein, 123 aa, Artificial Sequence
  Designed peptide
AEVQLVESGGAVVQPGGSLRLSCEASGFPFTKFWMYWVRRAPGKGLEWVAFIDTTGTITNYASSVKGRFTISRDDARNMVYLQMNDLRPEDTAIYYCATGPPGSAWVVDFHSWGQGTQVTVSS

SEQ ID NO: 35 - protein, 123 aa, Artificial Sequence
  Designed peptide
AEVQLVESGGAVVQPGGSLRLSCEASGFPFTKFWMYWVRRAPGKGLEWVAFIDTTGTITNYASSVKGRFTISRDDARNMVYLQMNDLRPEDTAIYYCATGPPGSTWVVDFNSWGQGTQVTVSS

SEQ ID NO: 36 - protein, 123 aa, Artificial Sequence
  Designed peptide
AEVQLVESGGAVVQPGGSLRLSCEASGFPFTKFWMYWVRRAPGKGLEWVAFIDTTGTITNYASSVKGRFTISRDDARNMVYLQMNDLRPEDTAIYYCATCPPGSTWVVDFHSWGQGTQVTVSS

SEQ ID NO: 37 - protein, 123 aa, Artificial Sequence
  Designed peptide
AEVQLVESGGAVVQPGGSLRLSCEASGFPFTKFWMYWVRRAPGKGLEWVAFIDTTGTITNYASSVKGRFTISRDDARNMVYLQMNDLRPEDTAIYYCATGPPGSTWVVDFDSWGQGTQVTVSS

SEQ ID NO: 38 - protein, 123 aa, Artificial Sequence
  Designed peptide
AEVQLVESGGAVVQPGGSLRLSCAASGFPFTKFWMYWVRRAPGKGLEWVAFIDTTGTITNYASSVKGRFTISRDDARNMVYLQMNDLRPEDTAIYYCATGPPGSAWVVDFHSWGQGTQVTVSS

SEQ ID NO: 39 - protein, 123 aa, Artificial Sequence
  Designed peptide
AEVQLVESGGAFVQPGGSLRLSCEASGFPFTKFWMYWVRRAPGKGLEWVAFIDTTGTITNYASSVKGRFTISRDDARNMVYLQMNDLRPEDTAIYYCATGPPGSTWVVDFNSWGQGTQVTVSS

SEQ ID NO: 40 - protein, 123 aa, Artificial Sequence
  Designed peptide
AEVQLVESGGAVVQPGGSLRLSCEASGFPFTKFWMYWVRRAPGKGLEWVAFIDTTGTITNYASSVKGRFTISRDDARNMVYLQMNDLSPEDTAIYYCATGPPGSPWVVDFHSWGQGTQVTVSS

SEQ ID NO: 41 - DNA, 10 bp, Artificial Sequence
  Synthetic oligonucleotide
gggshhhhhh

SEQ ID NO: 42 - protein, 133 aa, Artificial Sequence
  Designed peptide
AEVQLVESGGAVVQPGGSLRLSCEASGFPFTKFWMYWVRRAPGKGLEWVAFIDTTGTITNYASSVKGRFTISRDDARNMVYLQMNDLRPEDTAIYYCATGPPGSTWVVDFHSWGQGTQVTVSSGGGSHHHHHH

SEQ ID NO: 43 - protein, 129 aa, Artificial Sequence
  Designed peptide
AEVQLVESGGGSVQAGGSLTLSCAASGFTFDDHAVGWFRQAPGKGLEWVSAISGDGYTTVYADSVKGRFTISRDNAKKTVYLQMNSLKAEDTAVYYCNAFRTDIVREYWGQGTQVTVSSGGGSHHHHHH

SEQ ID NO: 44 - DNA, 432 bp, Artificial Sequence
  Synthetic oligonucleotide
gcagctcttgcagcagcagaagttcaactggttgaatcaggcggagcagttgttcaacctggcggatcactgagactgtcatgcgaagcatcaggctttccgtttacgaaattttggatgtattgggttagacgcgcacctggcaaaggcctggaatgggttgcatttattgatacaacaggcacgattacgaattatgcatcatcagtcaaaggacgctttacaatttcaagagatgatgcacgcaatatggtctacctgcaaatgaatgatcttcgtccggaagatacagcgatctattattgcgcaacaggccctccgggatcaacatgggttgttgattttcattcatggggacaaggcacacaagttacagtttcatctggcggaggctcacatcatcaccatcatcattaatctattaaactagtt

SEQ ID NO: 45 - DNA, 420 bp, Artificial Sequence
  Synthetic oligonucleotide
gcagctcttgcagcagcagaagttcaactggttgaatcaggcggaggctcagttcaagcaggcggatcactgacactgtcatgcgcagcatcaggctttacatttgatgatcatgcagttggctggtttagacaagcacctggcaaaggcctggaatgggtttcagcaattagcggagatggctatacaacagtttatgcagattcagtcaaaggacgctttacaatttcacgcgataacgcgaaaaaaacggtctatctgcaaatgaatagcctgaaagcagaagatacagcggtctattattgcaatgcatttcgcacagatatcgtcagagaatattggggacaaggcacacaagttacagtttcatctggcggaggcagccatcaccatcatcatcattaatctattaaactagtt

SEQ ID NO: 46 - DNA, 31 bp, Artificial Sequence
  Synthetic oligonucleotide
gatccccgggaattcctgttataaaaaaagg

SEQ ID NO: 47 - DNA, 27 bp, Artificial Sequence
  Synthetic oligonucleotide
atgatgttaagaaagaaaacaaagcag

SEQ ID NO: 48 - DNA, 38 bp, Artificial Sequence
  Synthetic oligonucleotide
gaattcccggggatctaagaaaagtgattctgggagag

SEQ ID NO: 49 - DNA, 36 bp, Artificial Sequence
  Synthetic oligonucleotide
ctttcttaacatcatagtagttcaccaccttttccc

SEQ ID NO: 50 - DNA, 25 bp, Artificial Sequence
  Synthetic oligonucleotide
tgctgcaagagctgccggaaataaa

SEQ ID NO: 51 - DNA, 21 bp, Artificial Sequence
  Synthetic oligonucleotide
tctattaaactagttataggg